European Patent Application EP 4 400 587 A1, published July 17, 2024. Title: トランス型ポリイソプレノイドの製造方法、ベクター、形質転換生物、空気入りタイヤの製造方法及びゴム製品の製造方法. Applicant: 住友ゴム工業株式会社. The sequence listing filed with the application follows.

SEQUENCE LISTING (39 sequences)

SEQ ID NO: 1 - DNA, 1263 bp, Manilkara zapota
  source 1..1263: mol_type = genomic DNA
atgttattttccaggggattttctcggatttcgagaaccagcttgaatcgcagtcgatgcctcttttcatttgaccaccagcatcaactattgattccgcctaatcacttctactctccgagtgactccactgaaaaggctttgagtggcagagataattattccttgggttcatttgcctttcacggcattgcacggcaattttatcaccagagcagccctgtagtggaggagcaacaggatccattttcccttgttgaaaatgaactatctattcttgctaataggttgcggtcaatggtagttgctgaggtcccaaagcttgcctcagctgctgagtacttcttcaagatgggggtggaaggaaagagatttcgaccaactgttttattgttgatggcaacagctctaaatgtacatatacccggaccaggttctaatggggtggttgatgttctatcgatggaactacgtaaaaggcaacagtgcatagctgagataacagaaatgatccatgtggcaagccttctgcatgatgatgtgttggatgatgcggatacaagacgtggcatagggtcattaaactttgtgatggggaataagttagcagtattggctggagatttcctgctttccagagcttgtgtggcccttgcctctttgaagaacacagaggttgtatcattgctagcaactgtggtagaacatcttgttacaggcgagaccatgcaaatgagtaccacatctgatcaacgttgtagcatggaatattatttgcaaaagacctactataagactgcatcattgatttcaaacagctgcaaagcaattgcccttcttgcagggcaaactgcagaggtttcaatgttggcttatgaatatggaaagaatctgggattggcatatcagttaatagatgacgttctagattttacaggcacatcagcttcccttggaaagggttctttatctgacatccgccatggaattgtaactgctccaatattatatgccatcgaggagttcccacagttgcgtgaagttgttgaccgaggaattgacaacactgcagatgtagatcttgttcttgattaccttggaaaaagtcgtggaatacagagaacgagagagctagcagccaagcacgccaaccttgcctcagctgcaatcgactctcttcctgagagtgatgatgagggtgttcaaagatcaaggcgagcactgttagatctaactcacagagtcattacaagagcaaagtag

SEQ ID NO: 2 - protein, 420 aa, Manilkara zapota
MLFSRGFSRISRTSLNRSRCLFSFDHQHQLLIPPNHFYSPSDSTEKALSGRDNYSLGSFAFHGIARQFYHQSSPVVEEQQDPFSLVENELSILANRLRSMVVAEVPKLASAAEYFFKMGVEGKRFRPTVLLLMATALNVHIPGPGSNGVVDVLSMELRKRQQCIAEITEMIHVASLLHDDVLDDADTRRGIGSLNFVMGNKLAVLAGDFLLSRACVALASLKNTEVVSLLATVVEHLVTGETMQMSTTSDQRCSMEYYLQKTYYKTASLISNSCKAIALLAGQTAEVSMLAYEYGKNLGLAYQLIDDVLDFTGTSASLGKGSLSDIRHGIVTAPILYAIEEFPQLREVVDRGIDNTADVDLVLDYLGKSRGIQRTRELAAKHANLASAAIDSLPESDDEGVQRSRRALLDLTHRVITRAK

SEQ ID NO: 3 - DNA, 1422 bp, Manilkara zapota
  source 1..1422: mol_type = genomic DNA
atggccttgaacctttttcaaaaccccatcactctttgtaaaaaccttgttaaatatgtgacttttcttctcatacaataccttctgaagtttcttattgaagagaatcgagcagatttgggtacaatatggaaagctttaagcgcaattccaattccaaacagtgatccgaaactgttcaaccgtccgaacaaggcagcagcgccaccaccaccgccgttgaagaagcagttccagaaggcggcaaccaccgaacactggctgctttcgcttgtcctaaacccagtcagttcatgtacaaatctcatctccattctcaaaagtcttgtcctaaacccagtcagcacttccaaaaatctaatcatctccctcgtcaaacacgttgctcagaaattcattcctggtgaagtactcgagaagaacttgctgccgccatggttgtcatcctcatcacctgattcaatacacccttctctagcccatgtaatcagcaacatcaagtccttcgagctcgaggacaaggctttgcatggaggtgaattcgacgaatacatggattccatgaacaaacaagtgaacaaggcactggatggactagtacccatgaagcatccagaaaaggttcacgaggcgatgagatactcccttttagcgggtgggaagcgagtgcgcccaatactgtgcattgcttcgtgccgattggtcggcggagacgaatcatcggcgttgccaatggcgtgtgcggtggagatcattcacaccgcttcgttgattgtggatgatcttccgtgcatggacaacgacgatctcaggcgaggcaaacccgcgagccacaaaatgtttggggaacaagtctcgattctttccagcgctggccttttcgctcttgcctttcagcatgtagccgctgcggagtacccagatatggtatcagttgatcgagtgattcgaggcattgttgagctggcttcggcgttggggacggaagggcttgttgggggccagtttatggacttggatagcgaaggaaaagatattagtgagaaagaactagagtacttgcatgtgaataaaacctcaaagctcttggaagcgtcggttgtttgtggagccatagttggaggggctagtgaggcagatatagagaaactaaggaaatatgcgaggctaatagggttgttgtttcaagtggtggatgatattctggatgtcacacaatccacagagaagctggggaagactgctgccaaggatttggtcagcaataaggccactttccccaagcttatgggtctcgacaatgccaagaaattcgccaacaagttggtcgaggaagccattcaagagattgctcactttgatgctgcaaaagctgctccgttgtaccatatcgctcattacattaataaccgtcaatattaa

SEQ ID NO: 4 - protein, 473 aa, Manilkara zapota
MALNLFQNPITLCKNLVKYVTFLLIQYLLKFLIEENRADLGTIWKALSAIPIPNSDPKLFNRPNKAAAPPPPPLKKQFQKAATTEHWLLSLVLNPVSSCTNLISILKSLVLNPVSTSKNLIISLVKHVAQKFIPGEVLEKNLLPPWLSSSSPDSIHPSLAHVISNIKSFELEDKALHGGEFDEYMDSMNKQVNKALDGLVPMKHPEKVHEAMRYSLLAGGKRVRPILCIASCRLVGGDESSALPMACAVEIIHTASLIVDDLPCMDNDDLRRGKPASHKMFGEQVSILSSAGLFALAFQHVAAAEYPDMVSVDRVIRGIVELASALGTEGLVGGQFMDLDSEGKDISEKELEYLHVNKTSKLLEASVVCGAIVGGASEADIEKLRKYARLIGLLFQVVDDILDVTQSTEKLGKTAAKDLVSNKATFPKLMGLDNAKKFANKLVEEAIQEIAHFDAAKAAPLYHIAHYINNRQY

SEQ ID NO: 5 - DNA, 768 bp, Chlamydomonas
  source 1..768: mol_type = genomic DNA
atggccgagtctgctggaaagcctctgaagcaccttgagtttgtgcacacctacgcgcacaagtttgcgagtggtgccgcttacgttgagggcggctaccagaaggccaagacctatgttcccgcggtcgctcagccctacatcgccaaagccgaggagacctgcctagcatacgccgctcctcttgcgacaaaggcgacggaccacgcagagaagattctccggagcaccgacgcacagctggacgcgctgtacgcggcctccgccagctggctgagcagctcccagaagctggccgactccaacatcgcggccttcaggggcgccgccgacaagtactacgacctggtcaagtccactgcgcagcacgtgacgtccaagctgcccaccgacctgtcggtggccaaggcccgcgagctgctgtcggcctcgctggagcaggccaaggctctggctgacccggacgctgcggtggcggcggcgctggatgcctggaccaagttcgcagccatcccggcggttgccaaggtgctgtccgccgcctccccgctgacgggcaagggcgtggcggccttcacggcggcacacgacctcctggtgcactcggcgctgtaccgctacggcgtgtcggtgggcgcctccaccctgggctgggccaccagcaccaccccctacaagttgagcgcggcttacctgtacccgctggtgcagcccgtggcggaccccgcgctggacaagcggagggccgccgtgcaacccggcccctag

SEQ ID NO: 6 - DNA, 948 bp, Manilkara zapota
  source 1..948: mol_type = genomic DNA
ctggcacatgttattagcaacatcaaatcctttgagctggaagataaagcactgcatggtggtgaatttgatgagtatatggacagcatgaacaaacaggttaataaagccctggatggtctggttccgatgaaacatccggaaaaagttcatgaagcaatgcgttatagcctgctggcaggcggtaaacgtgttcgtccgattctgtgtattgcaagctgtcgtctggttggtggtgatgaaagcagcgcactgccgatggcatgtgcagttgaaattattcataccgcaagcctgattgttgatgatctgccgtgtatggataatgatgacctgcgtcgtggtaaaccggcaagccataaaatgtttggtgaacaggttagtattctgagcagcgcaggtctgtttgcactggcatttcagcatgttgcagcagcagaatatcctgatatggttagcgttgatcgtgtgattcgtggtattgttgaactggcaagcgcactgggcaccgaaggcctggttggcggtcagtttatggatctggatagcgaaggtaaagatatcagcgaaaaagaactggaatatctgcacgtgaacaaaaccagcaaactgctggaagcaagcgttgtttgtggtgcaattgttggtggcgcaagcgaagcagatattgaaaaactgcgtaaatatgcccgtctgattggtctgctgtttcaggttgtggatgatattctggatgttacccagagcaccgaaaaactgggcaaaaccgcagccaaagatctggttagcaataaagcaacctttcctaaactgatgggccttgataatgccaaaaaattcgccaataaactggtggaagaggccattcaagaaatcgcacattttgatgcagcaaaagccgcaccgctgtatcatattgcacattatatcaataaccgccagtattaa

SEQ ID NO: 7 - DNA, 23 bp, synthetic construct
  misc_feature 1..23: note = PRIMER-1
  source 1..23: mol_type = other DNA
atgttattttccaggggattttc

SEQ ID NO: 8 - DNA, 25 bp, synthetic construct
  misc_feature 1..25: note = PRIMER-2
  source 1..25: mol_type = other DNA
ctactttgctcttgtaatgactctg

SEQ ID NO: 9 - DNA, 23 bp, synthetic construct
  misc_feature 1..23: note = PRIMER-3
  source 1..23: mol_type = other DNA
cgactggagcacgaggacactga

SEQ ID NO: 10 - DNA, 27 bp, synthetic construct
  misc_feature 1..27: note = PRIMER-4
  source 1..27: mol_type = other DNA
cttggggaaagtggccttattgctgac

SEQ ID NO: 11 - DNA, 26 bp, synthetic construct
  misc_feature 1..26: note = PRIMER-5
  source 1..26: mol_type = other DNA
ggacactgacatggactgaaggagta

SEQ ID NO: 12 - DNA, 27 bp, synthetic construct
  misc_feature 1..27: note = PRIMER-6
  source 1..27: mol_type = other DNA
ctgcctcactagcccctccaactatgg

SEQ ID NO: 13 - DNA, 38 bp, synthetic construct
  misc_feature 1..38: note = PRIMER-7
  source 1..38: mol_type = other DNA
tcagggcggatatctcgagatggccttgaacctttttc

SEQ ID NO: 14 - DNA, 47 bp, synthetic construct
  misc_feature 1..47: note = PRIMER-8
  source 1..47: mol_type = other DNA
ctagtgcggccgcggtaccattaatattgacggttattaatgtaatg

SEQ ID NO: 15 - DNA, 35 bp, synthetic construct
  misc_feature 1..35: note = PRIMER-9
  source 1..35: mol_type = other DNA
tatcgaaggtaggcatatggaggagcaacaggatc

SEQ ID NO: 16 - DNA, 44 bp, synthetic construct
  misc_feature 1..44: note = PRIMER-10
  source 1..44: mol_type = other DNA
cggatccctcgagggtaccctactttgctcttgtaatgactctg

SEQ ID NO: 17 - DNA, 39 bp, synthetic construct
  misc_feature 1..39: note = PRIMER-11
  source 1..39: mol_type = other DNA
catatcgaaggtaggcatatgctggcacatgttattagc

SEQ ID NO: 18 - DNA, 46 bp, synthetic construct
  misc_feature 1..46: note = PRIMER-12
  source 1..46: mol_type = other DNA
cggatccctcgagggtaccttaatactggcggttattgatataatg

SEQ ID NO: 19 - DNA, 41 bp, synthetic construct
  misc_feature 1..41: note = PRIMER-13
  source 1..41: mol_type = other DNA
catatcgaaggtaggcatatgttattttccaggggattttc

SEQ ID NO: 20 - DNA, 44 bp, synthetic construct; identical to SEQ ID NO: 16
  misc_feature 1..44: note = PRIMER-14
  source 1..44: mol_type = other DNA

SEQ ID NO: 21 - DNA, 25 bp, synthetic construct
  misc_feature 1..25: note = PRIMER-15
  source 1..25: mol_type = other DNA
catatgatggccttgaacctttttc

SEQ ID NO: 22 - DNA, 47 bp, synthetic construct; identical to SEQ ID NO: 14
  misc_feature 1..47: note = PRIMER-16
  source 1..47: mol_type = other DNA

SEQ ID NO: 23 - DNA, 29 bp, synthetic construct
  misc_feature 1..29: note = PRIMER-17
  source 1..29: mol_type = other DNA
agtcagatatctcatggccgagtctgctg

SEQ ID NO: 24 - DNA, 28 bp, synthetic construct
  misc_feature 1..28: note = PRIMER-18
  source 1..28: mol_type = other DNA
tgactggatcctcggggccgggttgcac

SEQ ID NO: 25 - DNA, 24 bp, synthetic construct
  misc_feature 1..24: note = PRIMER-19
  source 1..24: mol_type = other DNA
tgnsadggggsggsggsgggstag

SEQ ID NO: 26 - DNA, 34 bp, synthetic construct
  misc_feature 1..34: note = PRIMER-20
  source 1..34: mol_type = other DNA
agtcagatatctcatggccgagtctgctggaaag

SEQ ID NO: 27 - DNA, 36 bp, synthetic construct
  misc_feature 1..36: note = PRIMER-21
  source 1..36: mol_type = other DNA
ccgtcagcggaattaccggtggggccgggttgcacg

SEQ ID NO: 28 - DNA, 36 bp, synthetic construct
  misc_feature 1..36: note = PRIMER-22
  source 1..36: mol_type = other DNA
cgtgcaacccggccccaccggtaattccgctgacgg

SEQ ID NO: 29 - DNA, 31 bp, synthetic construct
  misc_feature 1..31: note = PRIMER-23
  source 1..31: mol_type = other DNA
tgactggatccgacccttgggtcgatcctcc

SEQ ID NO: 30 - DNA, 34 bp, synthetic construct; identical to SEQ ID NO: 26
  misc_feature 1..34: note = PRIMER-24
  source 1..34: mol_type = other DNA

SEQ ID NO: 31 - DNA, 31 bp, synthetic construct; identical to SEQ ID NO: 29
  misc_feature 1..31: note = PRIMER-25
  source 1..31: mol_type = other DNA

SEQ ID NO: 32 - DNA, 38 bp, synthetic construct
  misc_feature 1..38: note = PRIMER-26
  source 1..38: mol_type = other DNA
agtcacccgggctagcccatgtaatcagcaacatcaag

SEQ ID NO: 33 - DNA, 43 bp, synthetic construct
  misc_feature 1..43: note = PRIMER-27
  source 1..43: mol_type = other DNA
tgactgcggccgcgttaatattgacggttattaatgtaatgag

SEQ ID NO: 34 - DNA, 38 bp, synthetic construct; identical to SEQ ID NO: 32
  misc_feature 1..38: note = PRIMER-28
  source 1..38: mol_type = other DNA

SEQ ID NO: 35 - DNA, 43 bp, synthetic construct; identical to SEQ ID NO: 33
  misc_feature 1..43: note = PRIMER-29
  source 1..43: mol_type = other DNA

SEQ ID NO: 36 - DNA, 38 bp, synthetic construct
  misc_feature 1..38: note = PRIMER-30
  source 1..38: mol_type = other DNA
agtcacccgggatgttattttccaggggattttctcgg

SEQ ID NO: 37 - DNA, 39 bp, synthetic construct
  misc_feature 1..39: note = PRIMER-31
  source 1..39: mol_type = other DNA
tgactgcggccgcgctactttgctcttgtaatgactctg

SEQ ID NO: 38 - DNA, 30 bp, synthetic construct
  misc_feature 1..30: note = PRIMER-32
  source 1..30: mol_type = other DNA
agtcacccgggatggccttgaacctttttc

SEQ ID NO: 39 - DNA, 43 bp, synthetic construct; identical to SEQ ID NO: 33
  misc_feature 1..43: note = PRIMER-33
  source 1..43: mol_type = other DNA